European Patent Application EP 4 235 675 A1, published August 30, 2023. Title: A METHOD FOR PREDICTING HLA B-CELL EPITOPES CONSIDERING ALLELE-SPECIFIC SURFACE ACCESSIBLE RESIDUES. Applicant: PIRCHE AG. The sequence listing filed with the application follows.

SEQUENCE LISTING (10 sequences)

SEQ ID NO: 1 - protein, 23 aa, Homo sapiens
DMAAQITKRKWEAAHEAEQLRAY

SEQ ID NO: 2 - protein, 23 aa, Homo sapiens
DTAAQITQRKWEAAREAEQRRAY

SEQ ID NO: 3 - protein, 23 aa, Homo sapiens
DTAAQITQRKWEAARVAEQLRAY

SEQ ID NO: 4 - protein, 23 aa, Homo sapiens
DTAAQITQRKLEAARAAEQLRAY

SEQ ID NO: 5 - protein, 23 aa, Homo sapiens
DTAAQITQRKWEAAREAEQRRAY

SEQ ID NO: 6 - protein, 23 aa, Homo sapiens
DMAAQITKRKWEAVHAAEQRRVY

SEQ ID NO: 7 - protein, 23 aa, Homo sapiens
DTAAQITQRKWEAAREAEQRRAY

SEQ ID NO: 8 - protein, 23 aa, Homo sapiens
DTAAQITQRKWEAARVAEQLRAY

SEQ ID NO: 9 - protein, 23 aa, Homo sapiens
DTAAQITQRKLEAARAAEQLRAY

SEQ ID NO: 10 - protein, 23 aa, Homo sapiens
DTAAQITQRKWEAAREAEQRRAY